European Patent Specification EP 3 447 134 B1, published October 11, 2023. Title: Increased fungal resistance in crop plants. Applicant: KWS SAAT SE University of Bern University of Zurich. The sequence listing filed with the application follows.

SEQUENCE LISTING (65 sequences)

SEQ ID NO: 1 - DNA, 2004 bp, Zea mays
atggctgctcaccagcctcacctctccgtcctcctcctcgtcctcctcgctgcccatgtcgtctccacctccgcccatggcgagcctcctcttccgagcccttacaacacctccgcccatggcgagcctcctcttccgagcacttacaacgcctccatgtgctcgtcgttctggtgtggcggcgtcgagatccgctacccgttctatcttgccaacgcaatcgccgactacagcgggagctactactcctgcggctacaccgacttgagcgtttcctgcgaactcgaggtcgaggggtcgccgacgacctggacccctaccatccgtctcggcggcggcgactacaccgtcaagaacatctcctacctctacgaccagcagaccatctcactggcggacagagatgtgctcggaggcggcggctgccccgtcgtccgccacaacgtcagcttcgacgagacgtggctgcacctgcacaacgccagcgccttcgacaacctcaccttcttcttcggatgccactgggggccacggaatacaccgcctgaatttgccgactacaacatcagctgcgccgggttcaatactccaactatcagcggtggaaggtccttcgtgttcaagactggagatcttgacgaacaagaggagcaggagttggctttacactgcgacgaggttttctccgtgccagtgagaagagatgctctgcaggcgatcgtcagcaacttcagcctcacacgggacgggtacggcgaggtgcttaggcaggggttcgagttggaatggaatcggacatcggaggatcagtgtggccggtgcgagggatcgggctccggcggatggtgcgcctacagccagaagagagaattcctgggctgcttgtgcagcggagggaaggtgggcagcccgttctgcaaaccatcgagatcaaaaaggaaagaaggacctattgttggtgctgttgccgttgcattcctgtgtctagtcattctcacatgcttcttggcttgtagacatggttcgctgcccttcaaatcggagaacaaaccagggacaaggattgagtccttcctacagaagaacgagagtatacatccgaaaagatacacctacgcggacgtgaaaagaatgacaaaatccttcgctgtgaagctaggccaaggtgggtttggtgctgtatacaaaggcagcctccacgatggccgacaggtagcagtcaagatgctgaaggacacccaaggtgacggcgaggaattcatgaacgaggtggctagcatcagcaggacttctcatgtcaacgtcgtgacacttctagggttttgcttgcaagggtcgaaaagagcactgatctacgagtacatgcccaatggttcgctcgaaaggtatgccttcaccggtgacatgaacagtgagaatttgctaacctgggaaaggctatttgacatagcaattggcacggccagagggctcgaatacctacaccggggatgcaacactcggatcgtgcattttgacatcaagccacacaacatcctgttagaccaggatttctgtcctaagatctctgactttggactggccaagctatgtctgaacaaagagagcgctatctccattgctggcgcaagagggacgatagggtatatcgccccggaggtctactcaaagcaatttggaataataagcagcaagtctgatgtctatagctatgggatgatggtccttgagatggttggagcaagggacaggaatacaagcgcagatagtgaccatagcagccaatatttccctcagtggctttatgaacatttggacgactattgtgttggtgcttccgagattaatggtgagaccacagagctcgtgaggaagatgatagttgtaggtctgtggtgcatacaagtgattccgactgatcgaccaacaatgacgagagtcgtcgagatgttggaagggagcacaagtaatctagagttgccacccagagttctcttgagctga

SEQ ID NO: 2 - protein, 667 aa, Zea mays
MAAHQPHLSVLLLVLLAAHVVSTSAHGEPPLPSPYNTSAHGEPPLPSTYNASMCSSFWCGGVEIRYPFYLANAIADYSGSYYSCGYTDLSVSCELEVEGSPTTWTPTIRLGGGDYTVKNISYLYDQQTISLADRDVLGGGGCPVVRHNVSFDETWLHLHNASAFDNLTFFFGCHWGPRNTPPEFADYNISCAGFNTPTISGGRSFVFKTGDLDEQEEQELALHCDEVFSVPVRRDALQAIVSNFSLTRDGYGEVLRQGFELEWNRTSEDQCGRCEGSGSGGWCAYSQKREFLGCLCSGGKVGSPFCKPSRSKRKEGPIVGAVAVAFLCLVILTCFLACRHGSLPFKSENKPGTRIESFLQKNESIHPKRYTYADVKRMTKSFAVKLGQGGFGAVYKGSLHDGRQVAVKMLKDTQGDGEEFMNEVASISRTSHVNVVTLLGFCLQGSKRALIYEYMPNGSLERYAFTGDMNSENLLTWERLFDIAIGTARGLEYLHRGCNTRIVHFDIKPHNILLDQDFCPKISDFGLAKLCLNKESAISIAGARGTIGYIAPEVYSKQFGIISSKSDVYSYGMMVLEMVGARDRNTSADSDHSSQYFPQWLYEHLDDYCVGASEINGETTELVRKMIVVGLWCIQVIPTDRPTMTRVVEMLEGSTSNLELPPRVLLS

SEQ ID NO: 3 - DNA, 2004 bp, Artificial Sequence
  RLK1b - mutant Htn1
atggctgctcaccagcctcacctctccgtcctcctcctcgtcctcctcgctgcccatgtcgtctccacctccgcccatggcgagcctcctcttccgagcccttacaacacctccgcccatggcgagcctcctcttccgagcacttacaacgcctccatgtgctcgtcgttctggtgtggcggcgtcgagatccgctacccgttctatcttgccaacgcaatcgccgactacagcgggagctactactcctgcggctacaccgacttgagcgtttcctgcgaactcgaggtcgaggggtcgccgacgacctggacccctaccatccgtctcggcggcggcgactacaccgtcaagaacatctcctacctctacgaccagcagaccatctcactggcggacagagatgtgctcggaggcggcggctgccccgtcgtccgccacaacgtcagcttcgacgagacgtggctgcacctgcacaacgccagcgccttcgacaacctcaccttcttcttcggatgccactgggggccacggaatacaccgcctgaatttgccgactacaacatcagctgcgccgggttcaatactccaactatcagcggtggaaggtccttcgtgttcaagactggagatcttgacgaacaagaggagcaggagttggctttacactgcgacgaggttttctccgtgccagtgagaagagatgctctgcaggcgatcgtcagcaacttcagcctcacacgggacgggtacggcgaggtgcttaggcaggggttcgagttggaatggaatcggacatcggaggatcagtgtggccggtgcgagggatcgggctccggcggatggtgcgcctacagccagaagagagaattcctgggctgcttgtgcagcggagggaaggtgggcagcccgttctgcaaaccatcgagatcaaaaaggaaagaaggacctattgttggtgctgttgccgttgcattcctgtgtctagtcattctcacatgcttcttggcttgtagacatggttcgctgcccttcaaatcggagaacaaaccagggacaaggattgagtccttcctacagaagaacgagagtatacatccgaaaagatacacctacgcggacgtgaaaagaatgacaaaatccttcgctgtgaagctaggccaaggtgggtttggtgctgtatacaaaggcagcctccacgatggccgacaggtagcagtcaagatgctgaaggacacccaaggtgacggcgaggaattcatgaacgaggtggctagcatcagcaggacttctcatgtcaacgtcgtgacacttctagggttttgcttgcaagggtcgaaaagagcactgatctacgagtacatacccaatggttcgctcgaaaggtatgccttcaccggtgacatgaacagtgagaatttgctaacctgggaaaggctatttgacatagcaattggcacggccagagggctcgaatacctacaccggggatgcaacactcggatcgtgcattttgacatcaagccacacaacatcctgttagaccaggatttctgtcctaagatctctgactttggactggccaagctatgtctgaacaaagagagcgctatctccattgctggcgcaagagggacgatagggtatatcgccccggaggtctactcaaagcaatttggaataataagcagcaagtctgatgtctatagctatgggatgatggtccttgagatggttggagcaagggacaggaatacaagcgcagatagtgaccatagcagccaatatttccctcagtggctttatgaacatttggacgactattgtgttggtgcttccgagattaatggtgagaccacagagctcgtgaggaagatgatagttgtaggtctgtggtgcatacaagtgattccgactgatcgaccaacaatgacgagagtcgtcgagatgttggaagggagcacaagtaatctagagttgccacccagagttctcttgagctga

SEQ ID NO: 4 - protein, 667 aa, Artificial Sequence
  RLK1b - mutant Htn1
MAAHQPHLSVLLLVLLAAHVVSTSAHGEPPLPSPYNTSAHGEPPLPSTYNASMCSSFWCGGVEIRYPFYLANAIADYSGSYYSCGYTDLSVSCELEVEGSPTTWTPTIRLGGGDYTVKNISYLYDQQTISLADRDVLGGGGCPVVRHNVSFDETWLHLHNASAFDNLTFFFGCHWGPRNTPPEFADYNISCAGFNTPTISGGRSFVFKTGDLDEQEEQELALHCDEVFSVPVRRDALQAIVSNFSLTRDGYGEVLRQGFELEWNRTSEDQCGRCEGSGSGGWCAYSQKREFLGCLCSGGKVGSPFCKPSRSKRKEGPIVGAVAVAFLCLVILTCFLACRHGSLPFKSENKPGTRIESFLQKNESIHPKRYTYADVKRMTKSFAVKLGQGGFGAVYKGSLHDGRQVAVKMLKDTQGDGEEFMNEVASISRTSHVNVVTLLGFCLQGSKRALIYEYIPNGSLERYAFTGDMNSENLLTWERLFDIAIGTARGLEYLHRGCNTRIVHFDIKPHNILLDQDFCPKISDFGLAKLCLNKESAISIAGARGTIGYIAPEVYSKQFGIISSKSDVYSYGMMVLEMVGARDRNTSADSDHSSQYFPQWLYEHLDDYCVGASEINGETTELVRKMIVVGLWCIQVIPTDRPTMTRVVEMLEGSTSNLELPPRVLLS

SEQ ID NO: 5 - DNA, 2004 bp, Artificial Sequence
  RLK1d - mutant Htn1
atggctgctcaccagcctcacctctccgtcctcctcctcgtcctcctcgctgcccatgtcgtctccacctccgcccatggcgagcctcctcttccgagcccttacaacacctccgcccatggcgagcctcctcttccgagcacttacaacgcctccatgtgctcgtcgttctggtgtggcggcgtcgagatccgctacccgttctatcttgccaacgcaatcgccgactacagcgggagctactactcctgcggctacaccgacttgagcgtttcctgcgaactcgaggtcgaggggtcgccgacgacctggacccctaccatccgtctcggcggcggcgactacaccgtcaagaacatctcctacctctacgaccagcagaccatctcactggcggacagagatgtgctcggaggcggcggctgccccgtcgtccgccacaacgtcagcttcgacgagacgtggctgcacctgcacaacgccagcgccttcgacaacctcaccttcttcttcggatgccactgggggccacggaatacaccgcctgaatttgccgactacaacatcagctgcgccgggttcaatactccaactatcagcggtggaaggtccttcgtgttcaagactggagatcttgacgaacaagaggagcaggagttggctttacactgcgacgaggttttctccgtgccagtgagaagagatgctctgcaggcgatcgtcagcaacttcagcctcacacgggacgggtacggcgaggtgcttaggcaggggttcgagttggaatggaatcggacatcggaggatcagtgtggccggtgcgagggatcgggctccggcggatggtgcgcctacagccagaagagagaattcctgggctgcttgtgcagcggagggaaggtgggcagcccgttctgcaaaccatcgagatcaaaaaggaaagaaggacctattgttggtgctgttgccgttgcattcctgtgtctagtcattctcacatgcttcttggcttgtagacatggttcgctgcccttcaaatcggagaacaaaccagggacaaggattgagtccttcctacagaagaacgagagtatacatccgaaaagatacacctacgcggacgtgaaaagaatgacaaaatccttcgctgtgaagctaggccaaggtgggtttggtgctgtatacaaaggcagcctccacgatggccgacaggtagcagtcaagatgctgaaggacacccaaggtgacggcgaggaattcatgaacgaggtggctagcatcagcaggacttctcatgtcaacgtcgtgacacttctagggttttgcttgcaagggtcgaaaagagcactgatctacgagtacatgcccaatggttcgctcgaaaggtatgccttcaccggtgacatgaacagtgagaatttgctaacctgggaaaggctatttgacatagcaattggcacggccagagggctcgaatacctacaccgggaatgcaacactcggatcgtgcattttgacatcaagccacacaacatcctgttagaccaggatttctgtcctaagatctctgactttggactggccaagctatgtctgaacaaagagagcgctatctccattgctggcgcaagagggacgatagggtatatcgccccggaggtctactcaaagcaatttggaataataagcagcaagtctgatgtctatagctatgggatgatggtccttgagatggttggagcaagggacaggaatacaagcgcagatagtgaccatagcagccaatatttccctcagtggctttatgaacatttggacgactattgtgttggtgcttccgagattaatggtgagaccacagagctcgtgaggaagatgatagttgtaggtctgtggtgcatacaagtgattccgactgatcgaccaacaatgacgagagtcgtcgagatgttggaagggagcacaagtaatctagagttgccacccagagttctcttgagctga

SEQ ID NO: 6 - protein, 667 aa, Artificial Sequence
  RLK1d - mutant Htn1
MAAHQPHLSVLLLVLLAAHVVSTSAHGEPPLPSPYNTSAHGEPPLPSTYNASMCSSFWCGGVEIRYPFYLANAIADYSGSYYSCGYTDLSVSCELEVEGSPTTWTPTIRLGGGDYTVKNISYLYDQQTISLADRDVLGGGGCPVVRHNVSFDETWLHLHNASAFDNLTFFFGCHWGPRNTPPEFADYNISCAGFNTPTISGGRSFVFKTGDLDEQEEQELALHCDEVFSVPVRRDALQAIVSNFSLTRDGYGEVLRQGFELEWNRTSEDQCGRCEGSGSGGWCAYSQKREFLGCLCSGGKVGSPFCKPSRSKRKEGPIVGAVAVAFLCLVILTCFLACRHGSLPFKSENKPGTRIESFLQKNESIHPKRYTYADVKRMTKSFAVKLGQGGFGAVYKGSLHDGRQVAVKMLKDTQGDGEEFMNEVASISRTSHVNVVTLLGFCLQGSKRALIYEYMPNGSLERYAFTGDMNSENLLTWERLFDIAIGTARGLEYLHRECNTRIVHFDIKPHNILLDQDFCPKISDFGLAKLCLNKESAISIAGARGTIGYIAPEVYSKQFGIISSKSDVYSYGMMVLEMVGARDRNTSADSDHSSQYFPQWLYEHLDDYCVGASEINGETTELVRKMIVVGLWCIQVIPTDRPTMTRVVEMLEGSTSNLELPPRVLLS

SEQ ID NO: 7 - DNA, 2004 bp, Zea mays
atggctgctcacctaccacgcctccccgtcctcctcctcgtcctcctcgctgcccatgtcgtctccacctccgcccatgccgagcctcctcttccgagcccttacagcacctccgcccatggcgagcctcctcttccgagcacttacaacgtctccatgtgctcggaatcgttctggtgcggcggcgtcgaaatccgctacccgttctatcttgccaacgcaaccgccgactacagcgggagctactactcctgcggctacaccgacttgagcgtttcctgcaaactcgaggtcgaggggccgacgacgacatggacccctaccatccgtctcggcggcgacaactacaccgtcaagaacatcttgtacgactatcataccatctcactggcggacagcgatgtgctcggaggcggcgagtgccccgtcgtccaccacaacgtcagcttcgacgagacgtggctgcacaaccccagcgccttcgacaacctcaccttcttcttcggatgccactgggggccacgcgatacactgcctgaatttgccggcaacaacatcagctgcgccgggttcagtactccagctatcagcggtggaggctccttcgtgttcaagcctgaagatcttgacgaacatgcggagcaggagttggcttcacactgcgacgaggttttctccgtgccagtgagaagcgaggctctgcagcaggcgatcgtcagcaacctcagcctcggggacgggtacggcgagctgcttaggcaggggatcgagttggaatggaaacggacatcggaggatcagtgtggccagtgcgaggaatcgggctccggcggacggtgcgcctacagccagaagagagaattccttggctgcttctgcagcggagggaaggcgggcaacccgttctgcaaaccatcaagatcaacaaaaaggagagaagcagcatctattgttggtgctgttgccgttgcattcctgtgtctagtcattctcacatgcttcttggcttgtagacattgttcgctgcccttcaaatcgaagaacaaaccagggacaaggattgagtccttcctacagaagaacgagagtagtatacatccgaaaagatacacctacgcggacgtgaaaagaatgacaaaatccttcgctgtgaagctaggccaaggtgggtttggtgctgtatacaaaggcagcctccacgatggccgacaggtagcagtcaagatgctgaaggacacccaaggtgacggcgaggaattcatgaacgaggtggctagcatcagcaggacttctcatgtcaacgtcgtgacacttctagggttttgcttgcaagggtcgaaaagagcactgatctacgagtacatgcccaatggttcgctcgaaaggtatgccttcaccggtgacatgaacagtgagaatttgctaacctgggaaagactatttgacatagcgattggcacggccagagggctcgaatacctacaccggggatgcaacactcggatcgtgcattttgacatcaagccacacaacatcctgttagaccaggatttctgccctaagatctctgactttggactggccaagctatgtctgaacaaagagagcgctatctccattgctggcgcaagagggacgatagggtatatcgccccggaggtctactcaaagcaatttggaacgatcagcagcaagtctgatgtctatagctatgggatgatggtccttgagatggttggagcaagggacaggaatacaagcgcagatagtgaccatagcagccaatatttccctcagtggctttatgaacatttggacgactattgtgttggtgcttccgagattaatggtgagaccacagagctcgtgaggaagatgatagttgtaggtctgtggtgcatacaagtgattccgactgatcgaccaacaatgacgagagtcgtcgagatgttggaaggaagcacaagtaatctagagttgccacccagagttctcttgagctga

SEQ ID NO: 8 - protein, 667 aa, Zea mays
MAAHLPRLPVLLLVLLAAHVVSTSAHAEPPLPSPYSTSAHGEPPLPSTYNVSMCSESFWCGGVEIRYPFYLANATADYSGSYYSCGYTDLSVSCKLEVEGPTTTWTPTIRLGGDNYTVKNILYDYHTISLADSDVLGGGECPVVHHNVSFDETWLHNPSAFDNLTFFFGCHWGPRDTLPEFAGNNISCAGFSTPAISGGGSFVFKPEDLDEHAEQELASHCDEVFSVPVRSEALQQAIVSNLSLGDGYGELLRQGIELEWKRTSEDQCGQCEESGSGGRCAYSQKREFLGCFCSGGKAGNPFCKPSRSTKRREAASIVGAVAVAFLCLVILTCFLACRHCSLPFKSKNKPGTRIESFLQKNESSIHPKRYTYADVKRMTKSFAVKLGQGGFGAVYKGSLHDGRQVAVKMLKDTQGDGEEFMNEVASISRTSHVNVVTLLGFCLQGSKRALIYEYMPNGSLERYAFTGDMNSENLLTWERLFDIAIGTARGLEYLHRGCNTRIVHFDIKPHNILLDQDFCPKISDFGLAKLCLNKESAISIAGARGTIGYIAPEVYSKQFGTISSKSDVYSYGMMVLEMVGARDRNTSADSDHSSQYFPQWLYEHLDDYCVGASEINGETTELVRKMIVVGLWCIQVIPTDRPTMTRVVEMLEGSTSNLELPPRVLLS

SEQ ID NO: 9 - DNA, 11884 bp, Artificial Sequence
  ZmWAK-RLK1 plasmid
tacccgacgagtcagtaataaacggcgtcaaagtggttgcagccggcacacacgagtcgtgtttatcaactcaaagcacaaatacttttcctcaacctaaaaataaggcaattagccaaaaacaactttgcgtgtaaacaacgctcaatacacgtgtcattttattattagctattgcttcaccgccttagctttctcgtgacctagtcgtcctcgtcttttcttcttcttcttctataaaacaatacccaaagagctcttcttcttcacaattcagatttcaatttctcaaaatcttaaaaactttctctcaattctctctaccgtgatcaaggtaaatttctgtgttccttattctctcaaaatcttcgattttgttttcgttcgatcccaatttcgtatatgttctttggtttagattctgttaatcttagatcgaagacgattttctgggtttgatcgttagatatcatcttaattctcgattagggtttcatagatatcatccgatttgttcaaataatttgagttttgtcgaataattactcttcgatttgtgatttctatctagatctggtgttagtttctagtttgtgcgatcgaatttgtagattaatctgagtttttctgattaacactcgagtgcgggatcctctaagggcccatcacaagtttgtacaaaaaagcaggcttcatggctgctcaccagcctcacctctccgtcctcctcctcgtcctcctcgctgcccatgtcgtctccacctccgcccatggcgagcctcctcttccgagcccttacaacacctccgcccatggcgagcctcctcttccgagcacttacaacgcctccatgtgctcgtcgttctggtgtggcggcgtcgagatccgctacccgttctatcttgccaacgcaatcgccgactacagcgggagctactactcctgcggctacaccgacttgagcgtttcctgcgaactcgaggtcgaggggtcgccgacgacctggacccctaccatccgtctcggcggcggcgactacaccgtcaagaacatctcctacctctacgaccagcagaccatctcactggcggacagagatgtgctcggaggcggcggctgccccgtcgtccgccacaacgtcagcttcgacgagacgtggctgcacctgcacaacgccagcgccttcgacaacctcaccttcttcttcggatgccactgggggccacggaatacaccgcctgaatttgccgactacaacatcagctgcgccgggttcaatactccaactatcagcggtggaaggtccttcgtgttcaagactggagatcttgacgaacaagaggagcaggagttggctttacactgcgacgaggttttctccgtgccagtgagaagagatgctctgcaggcgatcgtcagcaacttcagcctcacacgggacgggtacggcgaggtgcttaggcaggggttcgagttggaatggaatcggacatcggaggatcagtgtggccggtgcgagggatcgggctccggcggatggtgcgcctacagccagaagagagaattcctgggctgcttgtgcagcggagggaaggtgggcagcccgttctgcaaaccatcgagatcaaaaaggaaagaaggacctattgttggtgctgttgccgttgcattcctgtgtctagtcattctcacatgcttcttggcttgtagacatggttcgctgcccttcaaatcggagaacaaaccagggacaaggattgagtccttcctacagaagaacgagagtatacatccgaaaagatacacctacgcggacgtgaaaagaatgacaaaatccttcgctgtgaagctaggccaaggtgggtttggtgctgtatacaaaggcagcctccacgatggccgacaggtagcagtcaagatgctgaaggacacccaaggtgacggcgaggaattcatgaacgaggtggctagcatcagcaggacttctcatgtcaacgtcgtgacacttctagggttttgcttgcaagggtcgaaaagagcactgatctacgagtacatgcccaatggttcgctcgaaaggtatgccttcaccggtgacatgaacagtgagaatttgctaacctgggaaaggctatttgacatagcaattggcacggccagagggctcgaatacctacaccggggatgcaacactcggatcgtgcattttgacatcaagccacacaacatcctgttagaccaggatttctgtcctaagatctctgactttggactggccaagctatgtctgaacaaagagagcgctatctccattgctggcgcaagagggacgatagggtatatcgccccggaggtctactcaaagcaatttggaataataagcagcaagtctgatgtctatagctatgggatgatggtccttgagatggttggagcaagggacaggaatacaagcgcagatagtgaccatagcagccaatatttccctcagtggctttatgaacatttggacgactattgtgttggtgcttccgagattaatggtgagaccacagagctcgtgaggaagatgatagttgtaggtctgtggtgcatacaagtgattccgactgatcgaccaacaatgacgagagtcgtcgagatgttggaagggagcacaagtaatctagagttgccacccagagttctcttgagccacccagctttcttgtacaaagtggtgatgggacgtccgcggagatctacgcgtgtcgactcgagatatccaactagtatggtgagcaagggcgaggagctgttcaccggggtggtgcccatcctggtcgagctggacggcgacgtaaacggccacaagttcagcgtgtccggcgagggcgagggcgatgccacctacggcaagctgaccctgaagttcatctgcaccaccggcaagctgcccgtgccctggcccaccctcgtgaccaccctgacctacggcgtgcagtgcttcagccgctaccccgaccacatgaagcagcacgacttcttcaagtccgccatgcccgaaggctacgtccaggagcgcaccatcttcttcaaggacgacggcaactacaagacccgcgccgaggtgaagttcgagggcgacaccctggtgaaccgcatcgagctgaagggcatcgacttcaaggaggacggcaacatcctggggcacaagctggagtacaactacaacagccacaacgtctatatcatggccgacaagcagaagaacggcatcaaggtgaacttcaagatccgccacaacatcgaggacggcagcgtgcagctcgccgaccactaccagcagaacacccccatcggcgacggccccgtgctgctgcccgacaaccactacctgagcacccagtccgccctgagcaaagaccccaacgagaagcgcgatcacatggtcctgctggagttcgtgaccgccgccgggatcactctcggcatggacgagctgtacaagttataagcggccatgctagagtccgcaaaaatcaccagtctctctctacaaatctatctctctctatttttctccagaataatgtgtgagtagttcccagataagggaattagggttcttatagggtttcgctcatgtgttgagcatataagaaacccttagtatgtatttgtatttgtaaaatacttctatcaataaaatttctaattcctaaaaccaaaatccagtgacctgcaggcatgcgacgtcgggccctctagaggatccccgggtaccgcgaattatcgatcatgagcggagaattaagggagtcacgttatgacccccgccgatgacgcgggacaagccgttttacgtttggaactgacagaaccgcaacgttgaaggagccactgagccgcgggtttctggagtttaatgagctaagcacatacgtcagaaaccattattgcgcgttcaaaagtcgcctaaggtcactatcagctagcaaatatttcttgtcaaaaatgctccactgacgttccataaattcccctcggtatccaattagagtctcatattcactctcaactcgatcgaggggatctaccatgagcccagaacgacgcccggccgacatccgccgtgccaccgaggcggacatgccggcggtctgcaccatcgtcaaccactacatcgagacaagcacggtcaacttccgtaccgagccgcaggaaccgcaggagtggacggacgacctcgtccgtctgcgggagcgctatccctggctcgtcgccgaggtggacggcgaggtcgccggcatcgcctacgcgggtccctggaaggcacgcaacgcctacgactggacggccgagtcgaccgtgtacgtctccccccgccaccagcggacgggactgggctccacgctctacacccacctgctgaagtccctggaggcacagggcttcaagagcgtggtcgctgtcatcgggctgcccaacgacccgagcgtgcgcatgcacgaggcgctcggatatgccccccgcggcatgctgcgggcggccggcttcaagcacgggaactggcatgacgtgggtttctggcagctggacttcagcctgccggtgccgccccgtccggtcctgcccgtcaccgaaatctgatgacccctagagtcaagcagatcgttcaaacatttggcaataaagtttcttaagattgaatcctgttgccggtcttgcgatgattatcatataatttctgttgaattacgttaagcatgtaataattaacatgtaatgcatgacgttatttatgagatgggtttttatgattagagtcccgcaattatacatttaatacgcgatagaaaacaaaatatagcgcgcaaactaggataaattatcgcgcgcggtgtcatctatgttactagatcgaccggcatgcaagctgataattcaattcggcgttaattcagtacattaaaaacgtccgcaatgtgttattaagttgtctaagcgtcaatttgtttacaccacaatatatcctgccaccagccagccaacagctccccgaccggcagctcggcacaaaatcaccactcgatacaggcagcccatcagtccgggacggcgtcagcgggagagccgttgtaaggcggcagactttgctcatgttaccgatgctattcggaagaacggcaactaagctgccgggtttgaaacacggatgatctcgcggagggtagcatgttgattgtaacgatgacagagcgttgctgcctgtgatcaattcgggcacgaacccagtggacataagcctgttcggttcgtaagctgtaatgcaagtagcgtatgcgctcacgcaactggtccagaaccttgaccgaacgcagcggtggtaacggcgcagtggcggttttcatggcttgttatgactgtttttttggggtacagtctatgcctcgggcatccaagcagcaagcgcgttacgccgtgggtcgatgtttgatgttatggagcagcaacgatgttacgcagcagggcagtcgccctaaaacaaagttaaacatcatgggggaagcggtgatcgccgaagtatcgactcaactatcagaggtagttggcgtcatcgagcgccatctcgaaccgacgttgctggccgtacatttgtacggctccgcagtggatggcggcctgaagccacacagtgatattgatttgctggttacggtgaccgtaaggcttgatgaaacaacgcggcgagctttgatcaacgaccttttggaaacttcggcttcccctggagagagcgagattctccgcgctgtagaagtcaccattgttgtgcacgacgacatcattccgtggcgttatccagctaagcgcgaactgcaatttggagaatggcagcgcaatgacattcttgcaggtatcttcgagccagccacgatcgacattgatctggctatcttgctgacaaaagcaagagaacatagcgttgccttggtaggtccagcggcggaggaactctttgatccggttcctgaacaggatctatttgaggcgctaaatgaaaccttaacgctatggaactcgccgcccgactgggctggcgatgagcgaaatgtagtgcttacgttgtcccgcatttggtacagcgcagtaaccggcaaaatcgcgccgaaggatgtcgctgccgactgggcaatggagcgcctgccggcccagtatcagcccgtcatacttgaagctagacaggcttatcttggacaagaagaagatcgcttggcctcgcgcgcagatcagttggaagaatttgtccactacgtgaaaggcgagatcaccaaggtagtcggcaaataatgtctagctagaaattcgttcaagccgacgccgcttcgcggcgcggcttaactcaagtcgttagatgcactaagcacataattgctcacagccaaactatcaggtcaagtctgcttttattatttttaagcgtgcataataagccctacacaaattgggagatatatcatgcatgaccaaaatcccttaacgtgagttttcgttccactgagcgtcagaccccgtagaaaagatcaaaggatcttcttgagatcctttttttctgcgcgtaatctgctgcttgcaaacaaaaaaaccaccgctaccagcggtggtttgtttgccggatcaagagctaccaactctttttccgaaggtaactggcttcagcagagcgcagataccaaatactgtccttctagtgtagccgtagttaggccaccacttcaagaactctgtagcaccgcctacatacctcgctctgctaatcctgttaccagtggctgctgccagtggcgataagtcgtgtcttaccgggttggactcaagacgatagttaccggataaggcgcagcggtcgggctgaacggggggttcgtgcacacagcccagcttggagcgaacgacctacaccgaactgagatacctacagcgtgagctatgagaaagcgccacgcttcccgaagggagaaaggcggacaggtatccggtaagcggcagggtcggaacaggagagcgcacgagggagcttccagggggaaacgcctggtatctttatagtcctgtcgggtttcgccacctctgacttgagcgtcgatttttgtgatgctcgtcaggggggcggagcctatggaaaaacgccagcaacgcggcctttttacggttcctggccttttgctggccttttgctcacatgttctttcctgcgttatcccctgattctgtggataaccgtattaccgcctttgagtgagctgataccgctcgccgcagccgaacgaccgagcgcagcgagtcagtgagcgaggaagcggaagagcgcctgatgcggtattttctccttacgcatctgtgcggtatttcacaccgcatatggtgcactctcagtacaatctgctctgatgccgcatagttaagccagtatacactccgctatcgctacgtgactgggtcatggctgcgccccgacacccgccaacacccgctgacgcgccctgacgggcttgtctgctcccggcatccgcttacagacaagctgtgaccgtctccgggagctgcatgtgtcagaggttttcaccgtcatcaccgaaacgcgcgaggcagggtgccttgatgtgggcgccggcggtcgagtggcgacggcgcggcttgtccgcgccctggtagattgcctggccctaggccagccatttttgagcggccagcggccgcgataggccgacgcgaagcggcggggcgtagggagcgcagcgaccgaagggtaggcgctttttgcagctcttcggctgtgcgctggccagacagttatgcacaggccaggcgggttttaagagttttaataagttttaaagagttttaggcggaaaaatcgccttttttctcttttatatcagtcacttacatgtgtgaccggttcccaatgtacggctttgggttcccaatgtacgggttccggttcccaatgtacggctttgggttcccaatgtacgtgctatccacaggaaagagaccttttcgacctttttcccctgctagggcaatttgccctagcatctgctccgtacattaggaaccggcggatgcttcgccctcgatcaggttgcggtagcgcatgactaggatcgggccagcctgccccgcctcctccttcaaatcgtactccggcaggtcatttgacccgatcagcttgcgcacggtgaaacagaacttcttgaactctccggcgctgccactgcgttcgtagatcgtcttgaacaaccatctggcttctgccttgcctgcggcgcggcgtgccaggcggtagagaaaacggccgatgccgggatcgatcaaaaagtaatcggggtgaaccgtcagcacgtccgggttcttgccttctgtgatctcgcggtacatccaatcagctagctcgatctcgatgtactccggccgcccggtttcgctctttacgatcttgtagcggctaatcaaggcttcaccctcggataccgtcaccaggcggccgttcttggccttcttcgtacgctgcatggcaacgtgcgtggtgtttaaccgaatgcaggtttctaccaggtcgtctttctgctttccgccatcggctcgccggcagaacttgagtacgtccgcaacgtgtggacggaacacgcggccgggcttgtctcccttcccttcccggtatcggttcatggattcggttagatgggaaaccgccatcagtaccaggtcgtaatcccacacactggccatgccggccggccctgcggaaacctctacgtgcccgtctggaagctcgtagcggatcacctcgccagctcgtcggtcacgcttcgacagacggaaaacggccacgtccatgatgctgcgactatcgcgggtgcccacgtcatagagcatcggaacgaaaaaatctggttgctcgtcgcccttgggcggcttcctaatcgacggcgcaccggctgccggcggttgccgggattctttgcggattcgatcagcggccgcttgccacgattcaccggggcgtgcttctgcctcgatgcgttgccgctgggcggcctgcgcggccttcaacttctccaccaggtcatcacccagcgccgcgccgatttgtaccgggccggatggtttgcgaccgtcacgccgattcctcgggcttgggggttccagtgccattgcagggccggcagacaacccagccgcttacgcctggccaaccgcccgttcctccacacatggggcattccacggcgtcggtgcctggttgttcttgattttccatgccgcctcctttagccgctaaaattcatctactcatttattcatttgctcatttactctggtagctgcgcgatgtattcagatagcagctcggtaatggtcttgccttggcgtaccgcgtacatcttcagcttggtgtgatcctccgccggcaactgaaagttgacccgcttcatggctggcgtgtctgccaggctggccaacgttgcagccttgctgctgcgtgcgctcggacggccggcacttagcgtgtttgtgcttttgctcattttctctttacctcattaactcaaatgagttttgatttaatttcagcggccagcgcctggacctcgcgggcagcgtcgccctcgggttctgattcaagaacggttgtgccggcggcggcagtgcctgggtagctcacgcgctgcgtgatacgggactcaagaatgggcagctcgtacccggccagcgcctcggcaacctcaccgccgatgcgcgtgcctttgatcgcccgcgacacgacaaaggccgcttgtagccttccatccgtgacctcaatgcgctgcttaaccagctccaccaggtcggcggtggcccatatgtcgtaagggcttggctgcaccggaatcagcacgaagtcggctgccttgatcgcggacacagccaagtccgccgcctggggcgctccgtcgatcactacgaagtcgcgccggccgatggccttcacgtcgcggtcaatcgtcgggcggtcgatgccgacaacggttagcggttgatcttcccgcacggccgcccaatcgcgggcactgccctggggatcggaatcgactaacagaacatcggccccggcgagttgcagggcgcgggctagatgggttgcgatggtcgtcttgcctgacccgcctttctggttaagtacagcgataaccttcatgcgttccccttgcgtatttgtttatttactcatcgcatcatatacgcagcgaccgcatgacgcaagctgttttactcaaatacacatcacctttttagacggcggcgctcggtttcttcagcggccaagctggccggccaggccgccagcttggcatcagacaaaccggccaggatttcatgcagccgcacggttgagacgtgcgcgggcggctcgaacacgtacccggccgcgatcatctccgcctcgatctcttcggtaatgaaaaacggttcgtcctggccgtcctggtgcggtttcatgcttgttcctcttggcgttcattctcggcggccgccagggcgtcggcctcggtcaatgcgtcctcacggaaggcaccgcgccgcctggcctcggtgggcgtcacttcctcgctgcgctcaagtgcgcggtacagggtcgagcgatgcacgccaagcagtgcagccgcctctttcacggtgcggccttcctggtcgatcagctcgcgggcgtgcgcgatctgtgccggggtgagggtagggcgggggccaaacttcacgcctcgggccttggcggcctcgcgcccgctccgggtgcggtcgatgattagggaacgctcgaactcggcaatgccggcgaacacggtcaacaccatgcggccggccggcgtggtggtgtcggcccacggctctgccaggctacgcaggcccgcgccggcctcctggatgcgctcggcaatgtccagtaggtcgcgggtgctgcgggccaggcggtctagcctggtcactgtcacaacgtcgccagggcgtaggtggtcaagcatcctggccagctccgggcggtcgcgcctggtgccggtgatcttctcggaaaacagcttggtgcagccggccgcgtgcagttcggcccgttggttggtcaagtcctggtcgtcggtgctgacgcgggcatagcccagcaggccagcggcggcgctcttgttcatggcgtaatgtctccggttctagtcgcaagtattctactttatgcgactaaaacacgcgacaagaaaacgccaggaaaagggcagggcggcagcctgtcgcgtaacttaggacttgtgcgacatgtcgttttcagaagacggctgcactgaacgtcagaagccgactgcactatagcagcggaggggttggatcaaagtactttaaagtactttaaagtactttaaagtactttgatcccgaggggaaccctgtggttggcatgcacatacaaatggacgaacggataaaccttttcacgcccttttaaatatccgttattctaataaacgctcttttctcttaggtttacccgccaatatatcctgtcaaacactgatagtttaaactgaaggcgggaaacgacaatctgatccaagctcaagctgctctagccaatacgcaaaccgcctctccccgcgcgttggccgattcattaatgcagctggcacgacaggtttcccgactggaaagcgggcagtgagcgcaacgcaattaatgtgagttagctcactcattaggcaccccaggctttacactttatgcttccggctcgtatgttgtgtggaattgtgagcggataacaatttcacacaggaaacagctatgaccatgattacgaattcgagctcgg

SEQ ID NO: 10 - DNA, 1044 bp, Zea mays
atggctttcgcgcccaaaacgtcctcctcctcctcgctctcctcggcgttgcaggcagctcagtcgccgccgctgctcctgaggcggatgtcgtcgaccgcaacaccgagacggaggtacgacgcggccgtcgtcgtcactaccaccaccactgctagagctgctgcggctgctgtcacggttcccgccgccccgccgcaggcgccggcgccggcgccggtgccgccaaagcaagcggcggcacccgccgagaggaggagccgtccggtgtcggacaccatggcggcgctcatggccaagggcaagacggcgttcatcccgtacataaccgccggcgaccccgacctagcgacgacggccgaggcgctgcggctgctggacggctgtggcgccgacgtcatcgagctgggcgtgccctgctcggacccctacatcgacgggcccatcatccaggcgtcggtggcgcgggctctggccagcggcaccaccatggacgccgtgctggagatgctgagggaggtgacgccggagctgtcgtgccccgtggtgctcctctcctactacaagcccatcatgtctcgcagcttggccgagatgaaagaggcgggggtccacggtcttatagtgcctgatctcccgtacgtggccgcgcactcgctgtggagtgaagccaagaacaacaacctggagctggtgctgctgacaacaccagccataccagaagacaggatgaaggagatcaccaaggcttcagaaggcttcgtctacctggtgagcgtgaacggagtgacaggtcctcgcgcaaacgtgaacccacgagtggagtcactcatccaggaggttaagaaggtgactaacaagcccgttgctgttggcttcggcatatccaagcccgagcacgtgaagcagattgcgcagtggggcgctgacggggtgatcatcggcagcgccatggtgaggcagctgggcgaagcggcttctcccaagcaaggcctgaggaggctggaggagtatgccaggggcatgaagaacgcgctgccatga

SEQ ID NO: 11 - protein, 347 aa, Zea mays
MAFAPKTSSSSSLSSALQAAQSPPLLLRRMSSTATPRRRYDAAVVVTTTTTARAAAAAVTVPAAPPQAPAPAPVPPKQAAAPAERRSRPVSDTMAALMAKGKTAFIPYITAGDPDLATTAEALRLLDGCGADVIELGVPCSDPYIDGPIIQASVARALASGTTMDAVLEMLREVTPELSCPVVLLSYYKPIMSRSLAEMKEAGVHGLIVPDLPYVAAHSLWSEAKNNNLELVLLTTPAIPEDRMKEITKASEGFVYLVSVNGVTGPRANVNPRVESLIQEVKKVTNKPVAVGFGISKPEHVKQIAQWGADGVIIGSAMVRQLGEAASPKQGLRRLEEYARGMKNALP

SEQ ID NO: 12 - DNA, 1182 bp, Zea mays
atgtacggcgccaccgactcgtgcttcgcgccctacggcgaccacttccgcaaggcgcggaagctggtcaccgtgcacctgctcaacgccagcaaggtgcggtcgcagcggcccgcgcgggaggaggaggtgcgcggcgcgctcgacagggtgcgccgcgccgccgccgcgcgggaggccctggacatgagcgagctcctgcactccttcgtcaacaacctcgtctgccgcgccgtctcgggcaagttctccatggaggaaggccgcaacaggctgttccgggagctcaccgacatcaacgcgggactcctcggagggttccacatccaggactacttccctagcctgggccggatcgagctcgtcaggaaggtggcgtgcgccaagaccaggcgcgtcaggaagcgctgggacgacctcctcgacaagctcatcgacgaccatgcggccaggatggcaacccatcaggacgaggacgacgataaggacttcatatacgtcttgctgtctcttcagaaggagtatggcctcaccagagaccatatcaaggctatcttgatagacatgttcgaggccggaaccgacacctcgtacatgacgttggagttcgccatgacggagctcatacggaagccacacctgatgaagaagctgcaggaagaagtgcggcggaacgtgccggcggggcaggagatggtcaccgaggacaacctccccggcatgacctacctcaaggccgtcatcaaggagacgctccgcctgcacccgccggtcccgctcctcctcccgcactactccctggacgcctgcgaggtcgccggctacaccatcccggccaacacccgcgtcgtcgtcaacgcctgggcgctcggccgccacagcggctactgggagcgcgagaacgagttcgtcccggagaggttcctcagcggggacgtggccggcggcgtcgacctcaagcccaacgagttccagttcctggcgttcgggtccggccggaggatgtgccccggggtccactcggcgtccgcgaccatcgaggcgatgctgtccaacctcatgtaccggttcgactggcagctgccggcggggatgaaggcggaggacgtggacatgaccgaggtgtttgggatcacggtctcgaggaaggagaagctgctcctagtcccacaggctgcgtga

SEQ ID NO: 13 - protein, 393 aa, Zea mays
MYGATDSCFAPYGDHFRKARKLVTVHLLNASKVRSQRPAREEEVRGALDRVRRAAAAREALDMSELLHSFVNNLVCRAVSGKFSMEEGRNRLFRELTDINAGLLGGFHIQDYFPSLGRIELVRKVACAKTRRVRKRWDDLLDKLIDDHAARMATHQDEDDDKDFIYVLLSLQKEYGLTRDHIKAILIDMFEAGTDTSYMTLEFAMTELIRKPHLMKKLQEEVRRNVPAGQEMVTEDNLPGMTYLKAVIKETLRLHPPVPLLLPHYSLDACEVAGYTIPANTRVVVNAWALGRHSGYWERENEFVPERFLSGDVAGGVDLKPNEFQFLAFGSGRRMCPGVHSASATIEAMLSNLMYRFDWQLPAGMKAEDVDMTEVFGITVSRKEKLLLVPQAA

SEQ ID NO: 14 - DNA, 1020 bp, Zea mays
atggcctccgcgatcaaggctgcatcgacctcctcccagtggtcttcttccccggcggcagtccactcgtcgccgttatcgaagcggctaccagctgcagtggccatgccggggcggcggaggtctgtggccactgtaagggcggtcgccgcggtagctccggctgccccggcggcgccggccaagctcaccgccggtgccggcggccgatgcctgccggtgtcgcagaccatgtccaggctcagggcgcagggcaagacggcgttcatcccgtacatcaccgccggcgacccggacctggcgacgacggcggaggcgctgcggctcctggacgcctgcggcgccgacgtcatcgagctcggcgttcccttctcggacccctacgccgacgggccggtcatccaggcgtcggcggcgcgggcactggcgagcggcacgacgccggacggcgtgctggcgatgctgaaggaggtgacgccggagctgtcctgccccgtggtgctcttctcctacttcaaccccatcgtgcggtggggcctggccgacttcgccgccgccgtcaaggaagccggcgtgcacggcctcatagttcccgacctcccgtatgggaactcgtgcgctctcactctcaggaccgaagccatcaagaacaacctcgagctggtgctgctcacaacaccatctacgccagcggacaggatggaggagataacacgagcttcacgaggattcgtctatctcgcgagcgtcaatggagttacaggtccacgcgcaaacgtgaacacacgtgtccagtctctcattcaggaggttaaacaggtcactgacatacccgtggctgtcgggtttggcatatcgaaacctgagcatgtaaagcagattgcagagtggggtgcagatggtgtgatcattggtagcgcaatggtgagacagttaggcgaagcagcctctcccaaagaaggattgaagaggctagagaaatacgccaggatcatgaagaacgcgctaccatgccagtga

SEQ ID NO: 15 - protein, 339 aa, Zea mays
MASAIKAASTSSQWSSSPAAVHSSPLSKRLPAAVAMPGRRRSVATVRAVAAVAPAAPAAPAKLTAGAGGRCLPVSQTMSRLRAQGKTAFIPYITAGDPDLATTAEALRLLDACGADVIELGVPFSDPYADGPVIQASAARALASGTTPDGVLAMLKEVTPELSCPVVLFSYFNPIVRWGLADFAAAVKEAGVHGLIVPDLPYGNSCALTLRTEAIKNNLELVLLTTPSTPADRMEEITRASRGFVYLASVNGVTGPRANVNTRVQSLIQEVKQVTDIPVAVGFGISKPEHVKQIAEWGADGVIIGSAMVRQLGEAASPKEGLKRLEKYARIMKNALPCQ

SEQ ID NO: 16 - DNA, 1125 bp, Zea mays
atggctccaacgaccgccaccaaggacgacagtggctacggcgacgagcgccggcgcgagctgcaggcgttcgacgacacgaagctgggggtgaaaggtctggtggactccggcgtcaagtccatcccgtccatcttccaccacccgccggaagccctgagcgacataatttctccggcgcctctgccgtcgtcgccaccctccggcgccgccatcccggtggtggacctctcggtgacgcggcgcgaggacctagtcgagcaggtgaggcacgcggccgggacggtgggcttcttctggctggtgaaccacggcgtggcggaggagctgatgggcggcatgctccgcggggtgcgccagttcaacgagggccccgtggaggcgaagcaggcgctctactccagggacctggctcgcaacctgcgcttcgcctccaacttcgacctcttcaaggccgctgcggccgactggcgcgacacgctcttctgcgaggtggctccgaacccgccgccgcgggaggagctgccggagccactgaggaacgtgatgctggagtacggcgcggcggtgacgaagctggcgcggttcgtgttcgagctgctgtccgagtccctcggcatgcccagcgaccacctgtacgagatggagtgcatgcagaacctgaacgtggtgtgccagtactacccgccgtgcccggagccgcaccgcaccgtgggcgtcaagaggcacacggaccctggcttcttcaccatcctcctgcaggacggcatgggcggcctgcaggtgcgcctcggcaacaacgggcagagcggcggctgctgggtggacatcgctccccggcctggggcgctcatggtcaacatcggtgatcttctgcagctcgtgaccaatgaccggttcaggagcgtggagcaccgggtgccagccaacaagagcagcgacacggcgagggtctccgtggcgtccttcttcaacacggacgtgaggaggtccgagaggatgtacggccccattccagaccccagcaagcccccgctgtacaggagcgtcagggcccgagacttcatcgcaaagttcaacaccataggactcgatggccgcgcgctcgaccacttcaggctctag

SEQ ID NO: 17 - protein, 374 aa, Zea mays
MAPTTATKDDSGYGDERRRELQAFDDTKLGVKGLVDSGVKSIPSIFHHPPEALSDIISPAPLPSSPPSGAAIPVVDLSVTRREDLVEQVRHAAGTVGFFWLVNHGVAEELMGGMLRGVRQFNEGPVEAKQALYSRDLARNLRFASNFDLFKAAAADWRDTLFCEVAPNPPPREELPEPLRNVMLEYGAAVTKLARFVFELLSESLGMPSDHLYEMECMQNLNVVCQYYPPCPEPHRTVGVKRHTDPGFFTILLQDGMGGLQVRLGNNGQSGGCWVDIAPRPGALMVNIGDLLQLVTNDRFRSVEHRVPANKSSDTARVSVASFFNTDVRRSERMYGPIPDPSKPPLYRSVRARDFIAKFNTIGLDGRALDHFRL

SEQ ID NO: 18 - DNA, 1128 bp, Zea mays
atggcactcatcatgcaggagagtagtagccatgatttgctccaagctcacgacgagctcttgcaccattccctgtgcttcgccaaatcgctcgcgctcgccgtggcgctggacctccgcatccccgacgcgatccaccaccacggcgccggcggcgccacccttctccagatcctcgccgagactgcgctccacccaagcaagcttcgcgcccttcgccgcctcatgcgcgtgctcaccgtcacgggcatcttcagcgtcgagcaaccaccagcaggtggtggtgataattcaaccgtccacacgtcggacgacgaagctgtcgtcgtctacaggttgacggcagcctcccgcttcctcgtcagcgacgaggtgagcacggcgaccttggctccctttgtgagtctggcgctccagcctatcgctgcctgtccgcacgccctgggtatctccgcgtggttccggcaggagcagcacgagccgtccccgtatggcctggcgttccggcagaccccaacgatctgggaacatgctgacgacgtaaacgccttgctgaacaaaggcatggccgcggacagccgcttcctcatgccaattgtgctgagggagtgcggcgagacgtttcgtgggatcgactcgttggttgacgtcggtggtggccatggtggcgccgccgccgccatcgccgccgccttcccccacctcaagtgcagcgtgcttgacctcccgcacgttgtcgccggtgctccgtctgatggcaacgtgcacttcgtcgcaggcaatatgtttgagagtattccacctgcaaccgctgttttcctcaagaaaactctacatgactggggtgacgatgagtgtgtcaagatattgaagaattgcaagcaagccatatctccacgggatgcaggtgggaaggtaataatcttggacgtggtagttggatataaacagtcaaacataaagcatcaagagacacaagttatgtttgatttgtatatgatggcggttaacggagttgagcgtgatgagcaagagtggaagaagatcttcattgaagctggattcaaagactacaaaattctacccgtcatcggtgacgtatcagtcatcatcgaggtctatccttga

SEQ ID NO: 19 - protein, 375 aa, Zea mays
MALIMQESSSHDLLQAHDELLHHSLCFAKSLALAVALDLRIPDAIHHHGAGGATLLQILAETALHPSKLRALRRLMRVLTVTGIFSVEQPPAGGGDNSTVHTSDDEAVVVYRLTAASRFLVSDEVSTATLAPFVSLALQPIAACPHALGISAWFRQEQHEPSPYGLAFRQTPTIWEHADDVNALLNKGMAADSRFLMPIVLRECGETFRGIDSLVDVGGGHGGAAAAIAAAFPHLKCSVLDLPHVVAGAPSDGNVHFVAGNMFESIPPATAVFLKKTLHDWGDDECVKILKNCKQAISPRDAGGKVIILDVVVGYKQSNIKHQETQVMFDLYMMAVNGVERDEQEWKKIFIEAGFKDYKILPVIGDVSVIIEVYP

SEQ ID NO: 20 - DNA, 1101 bp, Zea mays
atggcactcatgcaggagagcagccaggacttgctcgaagcgcacgacgagctcttccaccactgcctgtgcttcgccaaatcgctcgcgctcgccgtggcgcaggacctccgcatccccgacgcgatccaccaccacggaggcggcgccaccctccaccagatcctcgccgaggccgcgctccacccaagcaagcttcgcgccctacgccgcctgatgcgcgtgctcaccgtctcgggcgtcttcaccgtccagtattcttcaaccgtcgacgcgtcggacggagctgatgtcgtctacaggctgacggcagcctcccgcttcctcgtcagcgatagcgacgaggcgggcacggcgtccttggctccctttgcgaacctggcgctccaccctatcgccatctccccgcacgccgtgggcatctgcgcgtggttccggcaggagcagcacgacccgtccccgtacggcctggcgttccgccagatcccgaccatctgggagcatgctgacaacgtaaacgccctactgaacaaaggcttgctcgcggaaagccgcttcttgatgccaatcgtactcagggagtgcggagacgaggtgttccgtgggatcgactcgttggtcgacgtcggcggtgggcacggtggcgccgccgccaccatcgccgccgcattcccgcacgtcaagtgcagcgtgcttgacctcccgcacgttgtcgccggtgctccatccgatgcctgcgtgcagttcgttgcgggcaatatgttccacagtattccacctgcaaccgccgttttcttcaagacaactctatgtgactggggtgacgacgagtgcatcaagatattgaagaattgcaagcaagccatatctccacgggatgagggtgggaaggtgataatcatggacgtggtagtcgggtatgggcagtcaaacatgaagcgcctagagacacaagttatgtttgatttggttatgatggcggtcaatggagtcgagcgcgacgagcaagagtggaaggagatgttcattgaagctggattcaaagactacaaaatccgaccagtagctggcctcatgtcggtcatcgaggtctatccatga

SEQ ID NO: 21 - protein, 366 aa, Zea mays
MALMQESSQDLLEAHDELFHHCLCFAKSLALAVAQDLRIPDAIHHHGGGATLHQILAEAALHPSKLRALRRLMRVLTVSGVFTVQYSSTVDASDGADVVYRLTAASRFLVSDSDEAGTASLAPFANLALHPIAISPHAVGICAWFRQEQHDPSPYGLAFRQIPTIWEHADNVNALLNKGLLAESRFLMPIVLRECGDEVFRGIDSLVDVGGGHGGAAATIAAAFPHVKCSVLDLPHVVAGAPSDACVQFVAGNMFHSIPPATAVFFKTTLCDWGDDECIKILKNCKQAISPRDEGGKVIIMDVVVGYGQSNMKRLETQVMFDLVMMAVNGVERDEQEWKEMFIEAGFKDYKIRPVAGLMSVIEVYP

SEQ ID NO: 22 - DNA, 1122 bp, Zea mays
atggtgcagcaagccgcgaaggaggtgatcccgctgctgacgccttacaagatggggcagttcgagctctctcaccgggtggtgctggcgccgctgacgaggtgccgctcctacggcaacgtgccgcagccacacgccgccgtgtactactcgcaacgcgccaccaggggtggcctgctcatcgcggaggccacgggggtgtcggccaccgcgcaggggttcccggagtctcctggcatctggacgcaggagcaggtcgaggcgtggaagcccatcgtcgacgccgtccaccgcaagggcgccatcttcgtctgccagatctggcatgtgggcagggtctccaccaacgagctccagcccaacggcgacgcgcctatctcgagcacggacaagcagatctcccccgacgccaagtccggaacggcgtactcgaagccgcgccggctgcggaccgacgaggtccccgggatcgtcgacgacttcaggcgggccgcacggaacgcgatccaggctggtttcgacgccgtcgagatccacggcgcgcacgggtacctcctggagcagttcatgaaggacagctgcaacgaccgcacggaccagtacggcggcagcctggagaaccggtgccgtctcgccgtggaggtcgtggacgccgtcgtccgcgaggtgggcgcgcgccgcgtcggcatcaggctgtcgcccttcgtcgacttcgtggactgcgtggactcggacccggtggcgctcggccactacatggtgcagcagctcaacaggcatagcggcttgctctactgccacatggtggagccccgcattaccgcccacgggcgcaggcagatccctcacgggctcttgccgttccgaaaggcgtttcatggaacgttcatcgccgccggtgggtacgatcgggaggaaggcaacaaggtggtggcagaagggtatgctgacctcgtcgcgtatgggaagctgttcttggctaacccggacctgcctaggaggttcgagctggatgtggcactcaacaaatacgaccgctccaccttctacacgcaagatcctattgttggctacacagattaccctttctttgaagaagaagatggcaagaatgagaggtga

SEQ ID NO: 23 - protein, 373 aa, Zea mays
MVQQAAKEVIPLLTPYKMGQFELSHRVVLAPLTRCRSYGNVPQPHAAVYYSQRATRGGLLIAEATGVSATAQGFPESPGIWTQEQVEAWKPIVDAVHRKGAIFVCQIWHVGRVSTNELQPNGDAPISSTDKQISPDAKSGTAYSKPRRLRTDEVPGIVDDFRRAARNAIQAGFDAVEIHGAHGYLLEQFMKDSCNDRTDQYGGSLENRCRLAVEVVDAVVREVGARRVGIRLSPFVDFVDCVDSDPVALGHYMVQQLNRHSGLLYCHMVEPRITAHGRRQIPHGLLPFRKAFHGTFIAAGGYDREEGNKVVAEGYADLVAYGKLFLANPDLPRRFELDVALNKYDRSTFYTQDPIVGYTDYPFFEEEDGKNER

SEQ ID NO: 24 - DNA, 2595 bp, Zea mays
atgctgagcgggatcatcgacgggctgacgggggcgaacaagcatgcgcggctcaagggcacggtggtgctcatgcgcaagaacgtgctggacctcaacgacttcggcgccaccgtcgttgacagcatcagcgagttcctcggcaagggggtcacctgccagctcatcagctccaccctcgtcgacgccaacaacggcaaccgcgggcgggtcggggcggaggcgaacctggagcagtggctgacgagcctgccgtcgctgacgaccggcgagtccaagttcggcgtcacgttcgactgggaggtggagaagctgggagtgccgggggccgtcgtcgtcaagaacaaccacgccgccgagttcttcctcaagacaatcaccctcgacgacgtgcccggccgcggcgccgtcaccttcgtcgccaactcctgggtctaccccgcgggcaagtaccgctacaaccgcgtcttcttctccaacgatacgtacctgccaagccagatgccggcggcgctgaagccgtaccgcgacgacgagctccgcaacctccgcggcgacgaccagcagggcccctaccaggagcacgaccgcgtgtaccgctacgacgtctacaacgacctcggcgagcccgacggcggcaacccgcgccccatcctcggcggctccgccgaccacccgtacccgcgccgctgccgcacgggccgcaagcccaccaaaaccgaccccaactcggagagccgactgtcgctggtggagcagatctacgtgccgcgggacgagcgcttcggccacctcaagatgtccgacttcctgggctactccatcaaggccatcacgcagggcatcatcccggcggtgcgcacgtacgtggacaccaccccgggcgagttcgactccttccaggacatcatcaacctgtacgagggcgggatcaagctgcccaagatccaggcgctcgaggacatgcgcaagctcttcccgctccagctcgtcaaggacctcctccccgccggcggggactacctgctcaagctccccatcccacagatcatccaagaggacaagaacgcgtggaggaccgacgaggagttcgcgcgggaggtgctcgccggcgtcaacccgatggtgatcacgcgcctcacggagttcccgcccaagagcacgctggaccccagcaagtacggcgaccacaccagcacgatcacggcggagcacatcgagaagaacctcgagggcctcacggtgcagcaggcgctggacggcaacaggctctacatcctggaccaccacgaccgcttcatgccgttcctcatcgacgtcaacaacctggagggcaacttcatctacgccaccaggacgctcttcttcctgcgcggcgacggcaggctcgcgcccctcgccatcgagctcagcgagccgtacatcgacggggacctcaccgtggccaagagcaaggtctacacgccggcgtccagcggcgtcgaggcctgggtgtggcagctcgccaaggcctatgtcgccgtcaacgactctggctggcaccaactcgtcagccactggctgaacacccacgcggtgatggagccgttcgtgatcgcgacgaaccggcagctgagcgtgacgcacccggtgcacaagctcctgagctcgcacttccgcgacaccatgaccatcaacgcgctggcgcggcagacgctcatcaacggcggcggcatcttcgagatgaccgtcttcccgggcaagtacgcgctgggcatgtcctccgtggtgtacaagagctggaacttcaccgagcagggcctccccgccgacctcgtcaagaggggcgtggcggtggcggacccgtccagcccgtacaaggtgcggctgctgatcgaggactacccgtacgcgagcgacgggctggccatctggcacgccatcgagcagtgggtgggcgagtacctggccatctactaccccgacgacggcgcgctgcggggcgacgaggagctgcaggcgtggtggaaggaggtgcgcgaggtcgggcacggcgaccacaaggacgcgccctggtggcccaagatgcaggccgtgtcggagctcgccagcgcctgcaccaccatcatctggatcgcgtcggcgctccacgccgccgtcaacttcggccagtacccgtacgcggggtacctcccgaacaggcccacggtgagccggcgccggatgccggagcccggcagcaaggagtacgaggagctggagcgcgacccggagcgcggcttcatccacaccatcacgagccagatccagaccatcatcggcatctcgctcatcgagatcctctccaagcactcctccgacgaggtgtacctcggccagcgcgacacccccgagtggacctccgacgcccgggcgctggcggcgttcaagaggttcagcgacgcgctggtcaagatcgagggcaaggtggtgggcgagaaccgcgacccgcagctgaggaacaggaacggccccgccgagttcccctacatgctgctctatcccaacacctctgaccacagtggcgccgccgcagggctcactgccaagggcatccccaacagcatctccatctga

SEQ ID NO: 25 - protein, 864 aa, Zea mays
MLSGIIDGLTGANKHARLKGTVVLMRKNVLDLNDFGATVVDSISEFLGKGVTCQLISSTLVDANNGNRGRVGAEANLEQWLTSLPSLTTGESKFGVTFDWEVEKLGVPGAVVVKNNHAAEFFLKTITLDDVPGRGAVTFVANSWVYPAGKYRYNRVFFSNDTYLPSQMPAALKPYRDDELRNLRGDDQQGPYQEHDRVYRYDVYNDLGEPDGGNPRPILGGSADHPYPRRCRTGRKPTKTDPNSESRLSLVEQIYVPRDERFGHLKMSDFLGYSIKAITQGIIPAVRTYVDTTPGEFDSFQDIINLYEGGIKLPKIQALEDMRKLFPLQLVKDLLPAGGDYLLKLPIPQIIQEDKNAWRTDEEFAREVLAGVNPMVITRLTEFPPKSTLDPSKYGDHTSTITAEHIEKNLEGLTVQQALDGNRLYILDHHDRFMPFLIDVNNLEGNFIYATRTLFFLRGDGRLAPLAIELSEPYIDGDLTVAKSKVYTPASSGVEAWVWQLAKAYVAVNDSGWHQLVSHWLNTHAVMEPFVIATNRQLSVTHPVHKLLSSHFRDTMTINALARQTLINGGGIFEMTVFPGKYALGMSSVVYKSWNFTEQGLPADLVKRGVAVADPSSPYKVRLLIEDYPYASDGLAIWHAIEQWVGEYLAIYYPDDGALRGDEELQAWWKEVREVGHGDHKDAPWWPKMQAVSELASACTTIIWIASALHAAVNFGQYPYAGYLPNRPTVSRRRMPEPGSKEYEELERDPERGFIHTITSQIQTIIGISLIEILSKHSSDEVYLGQRDTPEWTSDARALAAFKRFSDALVKIEGKVVGENRDPQLRNRNGPAEFPYMLLYPNTSDHSGAAAGLTAKGIPNSISI

SEQ ID NO: 26 - DNA, 717 bp, Zea mays
atggccgccgcgctcaggtgcccggcctccgtcagggtctcgggccccgccgccgcggggctcgccaaggtgcgccaggcgtccagagtcgtcgcggtgagcggggcccggcagagccgcggcggcggcgtcgccgtgcgggcgtcgctgttctcgcccaagcccgcggcggccaaggacgcgcggccgaccaaggtgcaggagctgtacgtgtacgagatcaacgagcgggaccgcgagagccccgcgtacctgcgcctcagcgccaagcagacggagaacgcgctgggcgacctcgtccccttcaccaacaaggtgtacaacggcagcctggacaagcggctgggcgtcaccgcgggcatctgcgtgctcatccagcacgtccccgaccgcaacggcgaccgctacgaggccatctacagcttctacttcggagactacggccacatctcggtgcagggcccgtacctgacctacgaggagtcgtacctggcggtcaccggcggctccggcgtcttcgagggcgtctacggccaggtcaagctcaaccagatcgtcttccccttcaagatcttctacaccttctacctccggggcatcccggacctgcccagggacctgctctgcacgcccgtcccgccgtcgcccaccgtcgagcccacccccgccgccagggccgccgagccgcacgcatccctcgacaactacaccaactga

SEQ ID NO: 27 - protein, 238 aa, Zea mays
MAAALRCPASVRVSGPAAAGLAKVRQASRVVAVSGARQSRGGGVAVRASLFSPKPAAAKDARPTKVQELYVYEINERDRESPAYLRLSAKQTENALGDLVPFTNKVYNGSLDKRLGVTAGICVLIQHVPDRNGDRYEAIYSFYFGDYGHISVQGPYLTYEESYLAVTGGSGVFEGVYGQVKLNQIVFPFKIFYTFYLRGIPDLPRDLLCTPVPPSPTVEPTPAARAAEPHASLDNYTN

SEQ ID NO: 28 - DNA, 21 bp, Artificial Sequence
  Primer
taccatgttccctagggattg

SEQ ID NO: 29 - DNA, 20 bp, Artificial Sequence
  Primer
gtggcgcaatcactttaacc

SEQ ID NO: 30 - DNA, 20 bp, Artificial Sequence
  Primer
atctcgttggggatgtcttg

SEQ ID NO: 31 - DNA, 20 bp, Artificial Sequence
  Primer
agcaccgttcaaatgtctcc

SEQ ID NO: 32 - DNA, 20 bp, Artificial Sequence
  Primer
tattgttggtgctgttgccg

SEQ ID NO: 33 - DNA, 20 bp, Artificial Sequence
  Primer
ggactcaatccttgtccctg

SEQ ID NO: 34 - DNA, 20 bp, Artificial Sequence
  Primer
cccgagcacgtaaagcagat

SEQ ID NO: 35 - DNA, 20 bp, Artificial Sequence
  Primer
cttcatgcccctggcatact

SEQ ID NO: 36 - DNA, 23 bp, Artificial Sequence
  Primer
gacgaggacgacgataaggactt

SEQ ID NO: 37 - DNA, 25 bp, Artificial Sequence
  Primer
ggccatactccttctgaagagacag

SEQ ID NO: 38 - DNA, 20 bp, Artificial Sequence
  Primer
atggccgagctcatcaacaa

SEQ ID NO: 39 - DNA, 20 bp, Artificial Sequence
  Primer
tcgtcctcacctccgtctgt

SEQ ID NO: 40 - DNA, 20 bp, Artificial Sequence
  Primer
tgttcctccggatcatctgc

SEQ ID NO: 41 - DNA, 19 bp, Artificial Sequence
  Primer
aagaggctgtcccaccgct

SEQ ID NO: 42 - DNA, 20 bp, Artificial Sequence
  Primer
ccatttcgactgggaggtcc

SEQ ID NO: 43 - DNA, 20 bp, Artificial Sequence
  Primer
gtccatgctcaccttccagc

SEQ ID NO: 44 - DNA, 25 bp, Artificial Sequence
  Primer
aagttcaacaccataggactcgatg

SEQ ID NO: 45 - DNA, 25 bp, Artificial Sequence
  Primer
caggtagctagagcctgaagtggtc

SEQ ID NO: 46 - DNA, 20 bp, Artificial Sequence
  Primer
ggctgggttccgtgactaca

SEQ ID NO: 47 - DNA, 19 bp, Artificial Sequence
  Primer
gacctcgatgatggacggg

SEQ ID NO: 48 - DNA, 22 bp, Artificial Sequence
  Primer
ggaagaggatgaacgagctcaa

SEQ ID NO: 49 - DNA, 21 bp, Artificial Sequence
  Primer
gacccagcagattcatcgatg

SEQ ID NO: 50 - DNA, 19 bp, Artificial Sequence
  Primer
gggaccagttcggcaacat

SEQ ID NO: 51 - DNA, 18 bp, Artificial Sequence
  Primer
tgcccaccttccacacgt

SEQ ID NO: 52 - DNA, 20 bp, Artificial Sequence
  Primer
cagcaggtggtggtgataat

SEQ ID NO: 53 - DNA, 19 bp, Artificial Sequence
  Primer
agcgccagactcacaaagg

SEQ ID NO: 54 - DNA, 20 bp, Artificial Sequence
  Primer
gcccacccaagtaagcttcg

SEQ ID NO: 55 - DNA, 20 bp, Artificial Sequence
  Primer
agagacagcgataggatgga

SEQ ID NO: 56 - DNA, 20 bp, Artificial Sequence
  Primer
catcgtgtgccagtactacc

SEQ ID NO: 57 - DNA, 20 bp, Artificial Sequence
  Primer
accggtcattcgtcacaagc

SEQ ID NO: 58 - DNA, 20 bp, Artificial Sequence
  Primer
gcctcatagttcccgacctc

SEQ ID NO: 59 - DNA, 20 bp, Artificial Sequence
  Primer
gaatcctcgtgaagctcgtg

SEQ ID NO: 60 - DNA, 19 bp, Artificial Sequence
  Primer
cctcatgatgtgggtgcag

SEQ ID NO: 61 - DNA, 20 bp, Artificial Sequence
  Primer
atgcatgacaaggccagact

SEQ ID NO: 62 - DNA, 20 bp, Artificial Sequence
  Primer
aaaaacatgggacctcgtga

SEQ ID NO: 63 - DNA, 22 bp, Artificial Sequence
  Primer
attgcatgacgacaatgctaga

SEQ ID NO: 64 - DNA, 54 bp, Artificial Sequence
  Primer
ggggacaagtttgtacaaaaaagcaggcttcatggctgctcaccagcctcacct

SEQ ID NO: 65 - DNA, 54 bp, Artificial Sequence
  Primer
ggggaccactttgtacaagaaagctgggtggctcaagagaactctgggtggcaa